European Patent Application EP 4 428 150 A1, published September 11, 2024. Title: Antibody or antigen-binding fragment thereof. Applicant: Peptide Logic LLC. Application EP. The sequence listing filed with the application follows.

SEQUENCE LISTING (13 sequences)

SEQ ID NO: 1 - protein, 446 aa, synthetic construct
QVQLVQSGAEVKKPGASVKVSCKASGYTFSNFWIEWVRQAPGQRLEWMGEIFPGTGSTYYTEKFKVRVTITRDTSASTAYMELSSLRSEDTAVYYCARRGYSDSWFAHWGQGTLVTVSSASTKGPSVFPLAPCSRSTSESTAALGCLVKDYFPEPVTVSWNSGALTSGVHTFPAVLQSSGLYSLSSVVTVPSSSLGTKTYTCNVDHKPSNTKVDKRVESKYGPPCPPCPAPEFLGGPSVFLFPPKPKDTLMISRTPEVTCVVVDVSQEDPEVQFNWYVDGVEVHNAKTKPREEQFNSTYRVVSVLTVLHQDWLNGKEYKCKVSNKGLPSSIEKTISKAKGQPREPQVYTLPPSQEEMTKNQVSLTCLVKGFYPSDIAVEWESNGQPENNYKTTPPVLDSDGSFFLYSRLTVDKSRWQEGNVFSCSVMHEALHNHYTQKSLSLSLGK

SEQ ID NO: 2 - protein, 218 aa, synthetic construct
DIQMTQSPSSLSASVGDRVTITCRASESVDMYGKSFMHWYQQKPGKAPKLLIYRASTLESGVPSRFSGSGSGTDFTLTISSLQPEDFATYYCQQNVEAPLTFGGGTKVEIKRTVAAPSVFIFPPSDEQLKSGTASVVCLLNNFYPREAKVQWKVDNALQSGNSQESVTEQDSKDSTYSLSSTLTLSKADYEKHKVYACEVTHQGLSSPVTKSFNRGEC

SEQ ID NO: 3 - protein, 119 aa, synthetic construct
QVQLVQSGAEVKKPGASVKVSCKASGYTFSNFWIEWVRQAPGQRLEWMGEIFPGTGSTYYTEKFKVRVTITRDTSASTAYMELSSLRSEDTAVYYCARRGYSDSWFAHWGQGTLVTVSS

SEQ ID NO: 4 - protein, 111 aa, synthetic construct
DIQMTQSPSSLSASVGDRVTITCRASESVDMYGKSFMHWYQQKPGKAPKLLIYRASTLESGVPSRFSGSGSGTDFTLTISSLQPEDFATYYCQQNVEAPLTFGGGTKVEIK

SEQ ID NO: 5 - protein, 9 aa, synthetic construct
YTFSNFWIE

SEQ ID NO: 6 - protein, 17 aa, synthetic construct
EIFPGTGSTYYTEKFKV

SEQ ID NO: 7 - protein, 10 aa, synthetic construct
RGYSDSWFAH

SEQ ID NO: 8 - protein, 15 aa, synthetic construct
RASESVDMYGKSFMH

SEQ ID NO: 9 - protein, 7 aa, synthetic construct
RASTLES

SEQ ID NO: 10 - protein, 9 aa, synthetic construct
QQNVEAPLT

SEQ ID NO: 11 - protein, 161 aa, synthetic construct
EFDKRYTHGRGFITKAINSCHTSSLATPEDKEQAQQMNQKDFLSLIVSILRSWNEPLYHLVTEVRGMQEAPEAILSKAVEIEEQTKRLLEGMELIVSQVHPETKENEIYPVWSGLPSLQMADEESRLSAYYNLLHCLRRDSHKIDNYLKLLKCRIIHNNNC

SEQ ID NO: 12 - DNA, 1338 bp, synthetic construct
  source 1..1338: mol_type = other DNA
caagtgcagctggtgcagagcggcgccgaggtgaagaagcctggcgctagcgtgaaggtgagctgcaaggctagcggctacaccttcagcaacttctggatcgagtgggtgagacaagcccctggacagagactggagtggatgggcgagatcttccctggcaccggcagcacctactacaccgagaagttcaaggtgagagtgaccatcacaagagacacaagcgcgtccaccgcctacatggagctgagcagcctgagaagcgaggacaccgccgtgtactactgcgctagaagagggtattcagatagctggttcgcccactgggggcaaggcactctggtgaccgtgagcagcgctagcaccaaaggtcctagcgtgttccctctagccccttgcagcagaagcacaagcgagagcaccgccgccctgggctgcctggtgaaagactatttccctgagcctgtgaccgtgagttggaacagcggcgccctgacaagcggcgtgcacaccttccctgccgtgctgcagagcagcggcctgtacagcctgagcagcgtggtgaccgtgccaagcagcagcctgggcaccaagacctacacctgcaacgtggaccacaagcctagcaacaccaaggtggacaagagagtggagagcaagtacggtcctccgtgtcccccgtgccctgcccctgagttcctgggcggccctagcgtctttctgttcccacctaagcctaaggacaccctgatgatcagcagaacccctgaggtgacctgcgtggtggtggacgtgagccaagaggaccctgaggtgcagttcaactggtacgtggacggcgtggaggtgcacaacgccaagaccaagcctagagaggagcagttcaacagcacctacagagtggtgagcgtgctgaccgtgctgcaccaagactggctgaacggcaaggagtacaagtgcaaggtgagcaacaagggcctgcctagttccattgagaagaccatcagcaaggccaagggacagcctagagagcctcaagtgtacaccctgcctcctagccaagaggagatgaccaagaaccaagtgagcctgacctgcctggtaaaggggttctaccctagcgacatcgccgtggagtgggagagcaacggacagcctgagaacaactacaagaccacccctcctgtgctggacagcgacggcagcttcttcctgtacagcagactgaccgtggacaagagcagatggcaagagggcaacgtgttcagctgcagcgtgatgcacgaggccctgcacaaccactacacacagaagagcctgagcctgagcctgggcaag

SEQ ID NO: 13 - DNA, 654 bp, synthetic construct
  source 1..654: mol_type = other DNA
gacattcagatgacacagagccctagcagcctgagcgctagcgtgggcgacagagtgaccatcacctgcagagctagcgagagcgtggacatgtacggcaagagcttcatgcactggtatcagcagaagcctggcaaggcccctaagctgctgatctacagagctagcaccctggagagcggcgtgcctagcagattcagcggcagcggcagcggcaccgacttcaccctgaccatcagcagcctgcagcctgaggacttcgccacctactactgtcagcagaacgtggaggcccctctgaccttcggcggcggcaccaaggtggagatcaagagaaccgtggccgcccctagcgtgttcatcttccctcctagcgacgagcagctgaagagcggcaccgctagcgtggtgtgcctgctgaacaacttctaccctagagaggccaaggtgcagtggaaggtggacaacgccctgcagagcggcaacagccaagagagcgtgaccgagcaagacagcaaggacagcacctacagcctgagcagcaccctgaccctgagcaaggccgactacgagaagcacaaggtgtacgcctgcgaggtgacccaccaaggcctgagcagccctgtgaccaagagcttcaacagaggcgagtgc